European Patent Application EP 4 349 986 A1, published April 10, 2024. Title: Hetero nucleic acids comprising scpBNA or AmNA. Applicant: National University Corporation Tokyo Medical and Dental University Osaka University. The sequence listing filed with the application follows.

SEQUENCE LISTING (24 sequences)

SEQ ID NO: 1 - DNA, 16 bp, Artificial
  synthetic
  misc_feature (1)..(3), (14)..(16): scpBNA
atagtcactctggtga

SEQ ID NO: 2 - RNA, 16 nt, Artificial
  synthetic
ucaccagagugacuau

SEQ ID NO: 3 - DNA, 16 bp, Artificial
  synthetic
  misc_feature (1)..(3), (14)..(16): LNA
atagtcactctggtga

SEQ ID NO: 4 - DNA, 13 bp, Artificial
  synthetic
  misc_feature (1)..(3), (12)..(12): LNA
  misc_feature (13)..(13): 5-methylcytosine LNA
gttcactgaatgc

SEQ ID NO: 5 - RNA, 13 nt, Artificial
  synthetic
  misc_feature (1)..(2), (12)..(13): 2'-O-Me RNA
gcauucagugaac

SEQ ID NO: 6 - DNA, 13 bp, Artificial
  synthetic
  misc_feature (1)..(1), (12)..(12): LNA
  misc_feature (2)..(3): scpBNA
  misc_feature (13)..(13): 5-methylcytosine scpBNA
gttcactgaatgc

SEQ ID NO: 7 - DNA, 13 bp, Artificial
  synthetic
  misc_feature (1)..(1), (12)..(12): LNA
  misc_feature (2)..(3): AmNA
  misc_feature (13)..(13): 5-methylcytosine AmNA
gttcactgaatgc

SEQ ID NO: 8 - DNA, 14 bp, Artificial
  synthetic
  misc_feature (1)..(1), (14)..(14): LNA
  misc_feature (2)..(2), (13)..(13): 5-methylcytosine LNA
tcatggctgcagct

SEQ ID NO: 9 - RNA, 14 nt, Artificial
  synthetic
  misc_feature (1)..(2), (13)..(14): 2'-O-Me RNA
agcugcagccauga

SEQ ID NO: 10 - DNA, 14 bp, Artificial
  synthetic
  misc_feature (1)..(1), (14)..(14): scpBNA
  misc_feature (2)..(2), (13)..(13): 5-methylcytosine scpBNA
tcatggctgcagct

SEQ ID NO: 11 - DNA, 14 bp, Artificial
  synthetic
  misc_feature (1)..(1), (14)..(14): AmNA
  misc_feature (2)..(2), (13)..(13): 5-methylcytosine AmNA
tcatggctgcagct

SEQ ID NO: 12 - DNA, 14 bp, Artificial
  synthetic
  misc_feature (1)..(1), (13)..(13): LNA
  misc_feature (2)..(2), (14)..(14): 5-methylcytosine LNA
tcagtcatgacttc

SEQ ID NO: 13 - RNA, 14 nt, Artificial
  synthetic
  misc_feature (1)..(2), (13)..(14): 2'-O-Me RNA
gaagucaugacuga

SEQ ID NO: 14 - DNA, 14 bp, Artificial
  synthetic
  misc_feature (1)..(1), (13)..(13): scpBNA
  misc_feature (2)..(2), (14)..(14): 5-methylcytosine scpBNA
tcagtcatgacttc

SEQ ID NO: 15 - DNA, 14 bp, Artificial
  synthetic
  misc_feature (1)..(1), (13)..(13): AmNA
  misc_feature (2)..(2), (14)..(14): 5-methylcytosine AmNA
tcagtcatgacttc

SEQ ID NO: 16 - DNA, 14 bp, Artificial
  synthetic
  misc_feature (1)..(1), (13)..(13): LNA
  misc_feature (2)..(2), (14)..(14): 5-methylcytosine LNA
tcagtcatgacttc

SEQ ID NO: 17 - RNA, 14 nt, Artificial
  synthetic
  misc_feature (1)..(2), (13)..(14): 2'-O-Me RNA
gaagucaugacuga

SEQ ID NO: 18 - DNA, 14 bp, Artificial
  synthetic
  misc_feature (1)..(1), (13)..(13): scpBNA
  misc_feature (2)..(2), (14)..(14): 5-methylcytosine scpBNA
tcagtcatgacttc

SEQ ID NO: 19 - DNA, 6983 bp, Mus musculus
caggcattcaggcagcgagagcagagcagcgtagagcagcacagctgagctcgtgaggcaggagactcagcccgaggaaatcgcagataagtttttaattaaaaagattgagcagtaaaaagaattagaactctaaacttaagctaatagagtagcttatcgaaatattacttagtcttaataatctaagaagatcttaagagataacatgaaggcttatttaaacagtttgaaaaaggaaatgaggagaaaagtatttgtactgtataatggaggctgaccagagcagtttaggagattgtaaagggaggttttgtgaagttctaaaaggttctagtttgaaggtcggccttgtagattaaaacgaaggttacctaaatagaatctaagtggcatttaaaacagtaaagttgtagagaatagtttgaaaatgaggtgtagttttaaaagattgagaaaagtaggttaagttgacggccgttataaaaatccttcgactggcgcatgtacgtttgaaggcatgagttggaaacagggaagatggaagtgttaggctagccgggcgatggtggcgcacgcctttaatcctagcacttgggaggcagaggcaggcggatttctgagttcgaggccagcctggtctacagagtgagttccaggacagccagggctacacagagaaaccctgtcttgaaaaaacaaaaaggttaggctagtatttggagaaagaagattagaaaatggaagtgaaagacgaagaagacatacaggaaggtgaagaaaaagctgttagagaagataggaaaatagaagacaaagcatctttagaagacagaaaaggtacttaaaggcacaggtagtaggaagccgaagaatagaagatagaaagaagcaagatagaaaaacaaaatggaagttaagacaactttggatgccagcattcaagataggcaaagaagataagattgaggccaaaaggttggataagatataaagtcagaaggaaattatctttaaagccataagttcaaatttctgatggagcgagcagtttagaagagtctttagacagccacatacaagattgaagctagcaatcaaagctactaggactgaagtaaaaagttaaggcagaatgcctttgaagagttagaagaatattaaaagccttaacttgtagcttaattttgcttgatgacaaaaggacttttgataacagtttcaagattgtcagcattttgcattggacttgagctgaggtgcttttaaaatcctaacgactagcattggcagctgacccaggtctacacagaagtgcattcagtgaactaggaagacaggagcggcagacaggagtcccgaagccagtttggtgaagctaggaaggactgaggagccagcagcagcagtgcatggtgaagatagcccaggaaagagtgcggttcggtggaggaagctaggaagaaggagccatacggatgtggtggtgaagctgggaaagggttccaggatggtggagcgagagcgagttggtgatgaagctagctggcggcttggcttgtcaactgcgcggaggaggcgagcaggcattgtggagaggatagatagcggctcctagaccagcatgccagtgtgcaagaaaggctgcagggagagcatgcggtgcggtaacattccttgaggtcggcaacatggtggtggttttctgtaacttggatggtaacttgtttactttgtcttaatagttatgggggagttgtaggcttctgtgtaaagagatatatctggggctgtatgtaggcctttgcgggtgttgtaggtttttctttttcagggttatgtcctcttgcatcttgtcagaagcttttgagggctgactgccaaggcccagaaagaagaatggtagatggcaagttgtctttaaccgctcagaggggaatgaatggtagagccagcacaacctcccagttttgtaagacgttgtagtttgaacagatgacctaccacaagcctcactcctgtgtaggggaggtaattgggcaaagtgcttttgggggaatgggggcaaaatatattttgagttcttttccccttaggtctgtctagaatcctaaaggcagatgactcaagggaaccagaaaaaaggaaatccactctcaggataagcagagctcgccaggtttacagtttgtaggaagtagaggatggatgctagctttcacactgagtgtggaggagctggccatggcggaattgctggtagtttactctttccccctcccttaatgagatttgtaaaatcctaaacacttttacttgaaatatttgggagtggtcttaacagggaggagtgggtgggggaaacgttttttttctaagattttccacagatgctatagttgtgttgacacactgggttagagaaggcgtgtactgctatgctgttggcacgacaccttcagggactggagctgccttttgtccttggaagagttttcccagttgccgctgaagtcagcacagtgcggctttggttcacagtcacctcaggagaacctcaggagcttggctaggccagaggttgaagttaagttttacagcaccgtgatttaaaatatttcattaaaggggaggggtaaaacttagttggctgtggccttgtgtttgggtgggtgggggtgttaggtaattgtttagtttatgatttcagataatcataccagagaacttaaatatttggaaaaacaggaaatctcagctttcaagttggcaagtaactcccaatccagtttttgcttcttttttcctttttctttttttgaggcgggcagctaaggaaggttggttcctctgccggtccctcgaaagcgtagggcttgggggttggtctggtccactgggatgatgtgatgctacagtggggactcttctgaagctgttggatgaatatagattgtagtgtgtggttctcttttgaaatttttttcaggtgacttaatgtatcttaataactactataggaacaaaggaagtggctttaatgaccctgaaggaatttcttctggtgatagcttttatattatcaagtaagagatactatctcagttttgtataagcaagtctttttcctagtgtaggagaaatgattttccttgtgactaaacaagatgtaaaggtatgctttttttcttcttgtgcattgtatacttgtgtttatttgtaacttataatttaagaattatgataattcagcctgaatgtcttttagagggtgggcttttgttgatgagggaggggaaacctttttttttctgtagacctttttcagataacaccatctgagtcataaccagcctggcagtgtgatgacgtagatgcagagggagcagctccttggtgaatgagtgataagtaaaggcagaaaaaataatgtcatgtctccatggggaatgagcatgagccagagattgttcctactgatgaaaagctgcatatgcaaaaatttaagcaaatgaaagcaaccagtataaagttatggcaatacctttaaaagttatggcttatctaccaagctttatccacaaaagtaaagaattgatgaaaaacagtgaagatcaaatgttcatctcaaaactgcttttacaaaagcagaatagaaatgaagtgaaaatgctgcattaagcctggagtaaaaagaagctgagcttgttgagatgagtgggatcgagcggctgcgaggcggtgcagtgtgccaatgtttcgtttgcctcagacaggtttctcttcataagcagaagagttgcttcattccatctcggagcaggaaacagcagactgctgttgacagataagtgtaacttggatctgcagtattgcatgttagggatagataagtgccttttttctctttttccaaaaagacctgtagagctgttgaatgtttgcagctggcccctcttaggcagttcagaattttgagtagttttcccatccagcctcttaaaaattcctaagccttgcaccgatgggctttcatgatgggatagctaataggcttttgcatcgtaaacttcaacacaaaagcctacatgattaatgcctactttaattacattgcttacaagattaaggaatctttatcttgaagaccccatgaaagggatcattatgtgctgaaaattagatgttcatattgctaaaatttaaatgtgctccaatgtacttgtgcttaaaatcattaaattatacaaattaataaaatacttcactagagaatgtatgtatttagaaggctgtctccttatttaaataaagtcttgtttgttgtctgtagttagtgtgggcaattttggggggatgttcttctctaatcttttcagaaacttgacttcgaacacttaagtggaccagatcaggatttgagccagaagaccgaaattaactttaaggcaggaaagacaaattttattctccatgcagtgatgagcatttaataattgcaggcctggcatagaggccgtctaactaaggactaagtaccttaggcaggtgggagatgatggtcagagtaaaaggtaactacatattttgtttccagaaagtcaggggtctaatttgaccatggctaaacatctagggtaagacacttttcccccacatttccaaatatgcatgttgagtttaaatgcttacgatcatctcatccactttagccttttgtcacctcacttgagccacgagtggggtcaggcatgtgggtttaaagagttttcctttgcagagcctcatttcatccttcatggagctgctcaggactttgcatataagcgcttgcctctgtcttctgttctgctagtgagtgtgtgatgtgagaccttgcagtgagtttgtttttcctggaatgtggagggagggggggatggggcttacttgttctagctttttttttacagaccacacagaatgcaggtgtcttgacttcaggtcatgtctgttctttggcaagtaatatgtgcagtactgttccaatctgctgctattagaatgcattgtgacgcgactggagtatgattaaagaaagttgtgtttccccaagtgtttggagtagtggttgttggaggaaaagccatgagtaacaggctgagtgttgaggaaatggctctctgcagctttaagtaacccgtgtttgtgattggagccgagtccctttgctgtgctgccttaggtaaatgtttttgttcatttctggtgaggggggttgggagcactgaagcctttagtctcttccagattcaacttaaaatctgacaagaaataaatcagacaagcaacattcttgaagaaattttaactggcaagtggaaatgttttgaacagttccgtggtctttagtgcattatctttgtgtaggtgttctctctcccctcccttggtcttaattcttacatgcaggaacattgacaacagcagacatctatctattcaaggggccagagaatccagacccagtaaggaaaaatagcccatttactttaaatcgataagtgaagcagacatgccattttcagtgtggggattgggaagccctagttctttcagatgtacttcagactgtagaaggagcttccagttgaattgaaattcaccagtggacaaaatgaggacaacaggtgaacgagccttttcttgtttaagattagctactggtaatctagtgttgaatcctctccagcttcatgctggagcagctagcatgtgatgtaatgttggccttggggtggaggggtgaggtgggcgctaagcctttttttaagatttttcaggtacccctcactaaaggcactgaaggcttaatgtaggacagcggagccttcctgtgtggcaagaatcaagcaagcagtattgtatcgagaccaaagtggtatcatggtcggttttgattagcagtggggactaccctaccgtaacaccttgttggaattgaagcatccaaagaaaatacttgagaggccctgggcttgttttaacatctggaaaaaaggctgtttttatagcagcggttaccagcccaaacctcaagttgtgcttgcaggggagggaaaagggggaaagcgggcaaccagtttccccagcttttccagaatcctgttacaaggtctccccacaagtgatttctctgccacatcgccaccatgggcctttggcctaatcacagacccttcacccctcaccttgatgcagccagtagctggatccttgaggtcacgttgcatatcggtttcaaggtaaccatggtgccaaggtcctgtgggttgcaccagaaaaggccatcaattttccccttgcctgtaatttaacattaaaaccatagctaagatgttttatacatagcacctatgcagagtaaacaaaccagtatgggtatagtatgtttgataccagtgctgggtgggaatgtaggaagtcggatgaaaagcaagcctttgtaggaagttgttggggtgggattgcaaaaattctctgctaagactttttcaggtggacataacagacttggccaagctagcatcttagtggaagcagattcgtcagtagggttgtaaaggtttttcttttcctgagaaaacaaccttttgttttctcaggttttgctttttggcctttccctagctttaaaaaaaaaaaagcaaaagacgctggtggctggcactcctggtttccaggacggggttcaagtccctgcggtgtctttgcttgactcttatatcatgaggccattacatttttcttggagggttctaaaggctctgggtatggtagctgatatcactggaacactccccagcctcagtgttgaactcttgataattaactgcattgtctttcaggttatgcccaattcgtcttattacctctgagtcgacacacctcctactatttattgaatactttgattttatgaaataaaaactaaatatctctca

SEQ ID NO: 20 - DNA, 8779 bp, Homo sapiens
cgcagcctgcagcccgagacttctgtaaaggactggggccccgcaactggcctctcctgccctcttaagcgcagcgccattttagcaacgcagaagcccggcgccgggaagcctcagctcgcctgaaggcaggtcccctctgacgcctccgggagcccaggtttcccagagtccttgggacgcagcgacgagttgtgctgctatcttagctgtccttataggctggccattccaggtggtggtatttagataaaaccactcaaactctgcagtttggtcttggggtttggaggaaagcttttatttttcttcctgctccggttcagaaggtctgaagctcatacctaaccaggcataacacagaatctgcaaaacaaaaacccctaaaaaagcagacccagagcagtgtaaacacttctgggtgtgtccctgactggctgcccaaggtctctgtgtcttcggagacaaagccattcgcttagttggtctactttaaaaggccacttgaactcgctttccatggcgatttgccttgtgagcactttcaggagagcctggaagctgaaaaacggtagaaaaatttccgtgcgggccgtggggggctggcggcaactggggggccgcagatcagagtgggccactggcagccaacggcccccggggctcaggcggggagcagctctgtggtgtgggattgaggcgttttccaagagtgggttttcacgtttctaagatttcccaagcagacagcccgtgctgctccgatttctcgaacaaaaaagcaaaacgtgtggctgtcttgggagcaagtcgcaggactgcaagcagttgggggagaaagtccgccattttgccacttctcaaccgtccctgcaaggctggggctcagttgcgtaatggaaagtaaagccctgaactatcacactttaatcttccttcaaaaggtggtaaactatacctactgtccctcaagagaacacaagaagtgctttaagaggtattttaaaagttccgggggttttgtgaggtgtttgatgacccgtttaaaatatgatttccatgtttcttttgtctaaagtttgcagctcaaatctttccacacgctagtaatttaagtatttctgcatgtgtagtttgcattcaagttccataagctgttaagaaaaatctagaaaagtaaaactagaacctatttttaaccgaagaactactttttgcctccctcacaaaggcggcggaaggtgatcgaattccggtgatgcgagttgttctccgtctataaatacgcctcgcccgagctgtgcggtaggcattgaggcagccagcgcaggggcttctgctgagggggcaggcggagcttgaggaaaccgcagataagtttttttctctttgaaagatagagattaatacaactacttaaaaaatatagtcaataggttactaagatattgcttagcgttaagtttttaacgtaattttaatagcttaagattttaagagaaaatatgaagacttagaagagtagcatgaggaaggaaaagataaaaggtttctaaaacatgacggaggttgagatgaagcttcttcatggagtaaaaaatgtatttaaaagaaaattgagagaaaggactacagagccccgaattaataccaatagaagggcaatgcttttagattaaaatgaaggtgacttaaacagcttaaagtttagtttaaaagttgtaggtgattaaaataatttgaaggcgatcttttaaaaagagattaaaccgaaggtgattaaaagaccttgaaatccatgacgcagggagaattgcgtcatttaaagcctagttaacgcatttactaaacgcagacgaaaatggaaagattaattgggagtggtaggatgaaacaatttggagaagatagaagtttgaagtggaaaactggaagacagaagtacgggaaggcgaagaaaagaatagagaagatagggaaattagaagataaaaacatacttttagaagaaaaaagataaatttaaacctgaaaagtaggaagcagaagaaaaaagacaagctaggaaacaaaaagctaagggcaaaatgtacaaacttagaagaaaattggaagatagaaacaagatagaaaatgaaaatattgtcaagagtttcagatagaaaatgaaaaacaagctaagacaagtattggagaagtatagaagatagaaaaatataaagccaaaaattggataaaatagcactgaaaaaatgaggaaattattggtaaccaatttattttaaaagcccatcaatttaatttctggtggtgcagaagttagaaggtaaagcttgagaagatgagggtgtttacgtagaccagaaccaatttagaagaatacttgaagctagaaggggaagttggttaaaaatcacatcaaaaagctactaaaaggactggtgtaatttaaaaaaaactaaggcagaaggcttttggaagagttagaagaatttggaaggccttaaatatagtagcttagtttgaaaaatgtgaaggactttcgtaacggaagtaattcaagatcaagagtaattaccaacttaatgtttttgcattggactttgagttaagattattttttaaatcctgaggactagcattaattgacagctgacccaggtgctacacagaagtggattcagtgaatctaggaagacagcagcagacaggattccaggaaccagtgtttgatgaagctaggactgaggagcaagcgagcaagcagcagttcgtggtgaagataggaaaagagtccaggagccagtgcgatttggtgaaggaagctaggaagaaggaaggagcgctaacgatttggtggtgaagctaggaaaaaggattccaggaaggagcgagtgcaatttggtgatgaaggtagcaggcggcttggcttggcaaccacacggaggaggcgagcaggcgttgtgcgtagaggatcctagaccagcatgccagtgtgccaaggccacagggaaagcgagtggttggtaaaaatccgtgaggtcggcaatatgttgtttttctggaacttacttatggtaaccttttatttattttctaatataatgggggagtttcgtactgaggtgtaaagggatttatatggggacgtaggccgatttccgggtgttgtaggtttctctttttcaggcttatactcatgaatcttgtctgaagcttttgagggcagactgccaagtcctggagaaatagtagatggcaagtttgtgggttttttttttttacacgaatttgaggaaaaccaaatgaatttgatagccaaattgagacaatttcagcaaatctgtaagcagtttgtatgtttagttggggtaatgaagtatttcagttttgtgaatagatgacctgtttttacttcctcaccctgaattcgttttgtaaatgtagagtttggatgtgtaactgaggcgggggggagttttcagtatttttttttgtgggggtgggggcaaaatatgttttcagttctttttcccttaggtctgtctagaatcctaaaggcaaatgactcaaggtgtaacagaaaacaagaaaatccaatatcaggataatcagaccaccacaggtttacagtttatagaaactagagcagttctcacgttgaggtctgtggaagagatgtccattggagaaatggctggtagttactcttttttccccccacccccttaatcagactttaaaagtgcttaaccccttaaacttgttattttttacttgaagcattttgggatggtcttaacagggaagagagagggtgggggagaaaatgtttttttctaagattttccacagatgctatagtactattgacaaactgggttagagaaggagtgtaccgctgtgctgttggcacgaacaccttcagggactggagctgcttttatccttggaagagtattcccagttgaagctgaaaagtacagcacagtgcagctttggttcatattcagtcatctcaggagaacttcagaagagcttgagtaggccaaatgttgaagttaagttttccaataatgtgacttcttaaaagttttattaaaggggaggggcaaatattggcaattagttggcagtggcctgttacggttgggattggtggggtgggtttaggtaattgtttagtttatgattgcagataaactcatgccagagaacttaaagtcttagaatggaaaaagtaaagaaatatcaacttccaagttggcaagtaactcccaatgatttagtttttttccccccagtttgaattgggaagctgggggaagttaaatatgagccactgggtgtaccagtgcattaatttgggcaaggaaagtgtcataatttgatactgtatctgttttccttcaaagtatagagcttttggggaaggaaagtattgaactgggggttggtctggcctactgggctgacattaactacaattatgggaaatgcaaaagttgtttggatatggtagtgtgtggttctcttttggaatttttttcaggtgatttaataataatttaaaactactatagaaactgcagagcaaaggaagtggcttaatgatcctgaagggatttcttctgatggtagcttttgtattatcaagtaagattctattttcagttgtgtgtaagcaagtttttttttagtgtaggagaaatacttttccattgtttaactgcaaaacaagatgttaaggtatgcttcaaaaattttgtaaattgtttattttaaacttatctgtttgtaaattgtaactgattaagaattgtgatagttcagcttgaatgtctcttagagggtgggcttttgttgatgagggaggggaaactttttttttttctatagacttttttcagataacatcttctgagtcataaccagcctggcagtatgatggcctagatgcagagaaaacagctccttggtgaattgataagtaaaggcagaaaagattatatgtcatacctccattggggaataagcataaccctgagattcttactactgatgagaacattatctgcatatgccaaaaaattttaagcaaatgaaagctaccaatttaaagttacggaatctaccattttaaagttaattgcttgtcaagctataaccacaaaaataatgaattgatgagaaatacaatgaagaggcaatgtccatctcaaaatactgcttttacaaaagcagaataaaagcgaaaagaaatgaaaatgttacactacattaatcctggaataaaagaagccgaaataaatgagagatgagttgggatcaagtggattgaggaggctgtgctgtgtgccaatgtttcgtttgcctcagacaggtatctcttcgttatcagaagagttgcttcatttcatctgggagcagaaaacagcaggcagctgttaacagataagtttaacttgcatctgcagtattgcatgttagggataagtgcttatttttaagagctgtggagttcttaaatatcaaccatggcactttctcctgaccccttccctaggggatttcaggattgagaaatttttccatcgagcctttttaaaattgtaggacttgttcctgtgggcttcagtgatgggatagtacacttcactcagaggcatttgcatctttaaataatttcttaaaagcctctaaagtgatcagtgccttgatgccaactaaggaaatttgtttagcattgaatctctgaaggctctatgaaaggaatagcatgatgtgctgttagaatcagatgttactgctaaaatttacatgttgtgatgtaaattgtgtagaaaaccattaaatcattcaaaataataaactatttttattagagaatgtatacttttagaaagctgtctccttatttaaataaaatagtgtttgtctgtagttcagtgttggggcaatcttgggggggattcttctctaatctttcagaaactttgtctgcgaacactctttaatggaccagatcaggatttgagcggaagaacgaatgtaactttaaggcaggaaagacaaattttattcttcataaagtgatgagcatataataattccaggcacatggcaatagaggccctctaaataaggaataaataacctcttagacaggtgggagattatgatcagagtaaaaggtaattacacattttatttccagaaagtcaggggtctataaattgacagtgattagagtaatactttttcacatttccaaagtttgcatgttaactttaaatgcttacaatcttagagtggtaggcaatgttttacactattgaccttatatagggaagggagggggtgcctgtggggttttaaagaattttcctttgcagaggcatttcatccttcatgaagccattcaggattttgaattgcatatgagtgcttggctcttccttctgttctagtgagtgtatgagaccttgcagtgagtttatcagcatactcaaaatttttttcctggaatttggagggatgggaggagggggtggggcttacttgttgtagctttttttttttttacagacttcacagagaatgcagttgtcttgacttcaggtctgtctgttctgttggcaagtaaatgcagtactgttctgatcccgctgctattagaatgcattgtgaaacgactggagtatgattaaaagttgtgttccccaatgcttggagtagtgattgttgaaggaaaaaatccagctgagtgataaaggctgagtgttgaggaaatttctgcagttttaagcagtcgtatttgtgattgaagctgagtacattttgctggtgtatttttaggtaaaatgctttttgttcatttctggtggtgggaggggactgaagcctttagtcttttccagatgcaaccttaaaatcagtgacaagaaacattccaaacaagcaacagtcttcaagaaattaaactggcaagtggaaatgtttaaacagttcagtgatctttagtgcattgtttatgtgtgggtttctctctcccctcccttggtcttaattcttacatgcaggaacactcagcagacacacgtatgcgaagggccagagaagccagacccagtaagaaaaaatagcctatttactttaaataaaccaaacattccattttaaatgtggggattgggaaccactagttctttcagatggtattcttcagactatagaaggagcttccagttgaattcaccagtggacaaaatgaggaaaacaggtgaacaagctttttctgtatttacatacaaagtcagatcagttatgggacaatagtattgaatagatttcagctttatgctggagtaactggcatgtgagcaaactgtgttggcgtgggggtggaggggtgaggtgggcgctaagcctttttttaagatttttcaggtacccctcactaaaggcaccgaaggcttaaagtaggacaaccatggagccttcctgtggcaggagagacaacaaagcgctattatcctaaggtcaagagaagtgtcagcctcacctgatttttattagtaatgaggacttgcctcaactccctctttctggagtgaagcatccgaaggaatgcttgaagtacccctgggcttctcttaacatttaagcaagctgtttttatagcagctcttaataataaagcccaaatctcaagcggtgcttgaaggggagggaaagggggaaagcgggcaaccacttttccctagcttttccagaagcctgttaaaagcaaggtctccccacaagcaacttctctgccacatcgccaccccgtgccttttgatctagcacagacccttcacccctcacctcgatgcagccagtagcttggatccttgtgggcatgatccataatcggtttcaaggtaacgatggtgtcgaggtctttggtgggttgaactatgttagaaaaggccattaatttgcctgcaaattgttaacagaagggtattaaaaccacagctaagtagctctattataatacttatccagtgactaaaaccaacttaaaccagtaagtggagaaataacatgttcaagaactgtaatgctgggtgggaacatgtaacttgtagactggagaagataggcatttgagtggctgagagggcttttgggtgggaatgcaaaaattctctgctaagactttttcaggtgaacataacagacttggccaagctagcatcttagcggaagctgatctccaatgctcttcagtagggtcatgaaggtttttcttttcctgagaaaacaacacgtattgttttctcaggttttgctttttggcctttttctagcttaaaaaaaaaaaaagcaaaagatgctggtggttggcactcctggtttccaggacggggttcaaatccctgcggcgtctttgctttgactactaatctgtcttcaggactctttctgtatttctccttttctctgcaggtgctagttcttggagttttggggaggtgggaggtaacagcacaatatctttgaactatatacatccttgatgtataatttgtcaggagcttgacttgattgtatattcatatttacacgagaacctaatataactgccttgtctttttcaggtaatagcctgcagctggtgttttgagaagccctactgctgaaaacttaacaattttgtgtaataaaaatggagaagctctaaattgttgtggttcttttgtgaataaaaaaatcttgattggggaaaaaa

SEQ ID NO: 21 - DNA, 2534 bp, Mus musculus
ggaatcccgcgccgaactcgggggcgggctgcccgggccatggcgcataaagcctctggccacctgcagggctactgctgctccggccaccgccaggcacacaccttgctgctgagggagtctcggcttctgtcatctctgtggcctccgtcacctctgtctccgtctccttcaggtcctgagccccgagagccccttccgcgcacgcggacatgggcggcagctccagggcgcgctgggtggccttggggttgggcgccctggggctgctgtttgctgcgctcggcgttgtcatgatcctcatggtgccctccctcatcaagcagcaggtgctcaagaatgtccgcatagacccgagcagcctgtccttcgggatgtggaaggagatccccgtccctttctacttgtctgtctacttcttcgaagtggtcaacccaaacgaggtcctcaacggccagaagccagtagtccgggagcgtggaccctatgtctacagggagttcagacaaaaggtcaacatcaccttcaatgacaacgacaccgtgtccttcgtggagaaccgcagcctccatttccagcctgacaagtcgcatggctcagagagtgactacattgtactgcctaacatcttggtcctggggggctcgatattgatggagagcaagcctgtgagcctgaagctgatgatgaccttggcgctggtcaccatgggccagcgtgcttttatgaaccgcacagttggtgagatcctgtggggctatgacgatcccttcgtgcattttctcaacacgtacctcccagacatgcttcccataaagggcaaatttggcctgtttgttgggatgaacaactcgaattctggggtcttcactgtcttcacgggcgtccagaatttcagcaggatccatctggtggacaaatggaacggactcagcaagatcgattattggcattcagagcagtgtaacatgatcaatgggacttccgggcagatgtgggcacccttcatgacacccgaatcctcgctggaattcttcagcccggaggcatgcaggtccatgaagctgacctacaacgaatcaagggtgtttgaaggcattcccacgtatcgcttcacggcccccgatactctgtttgccaacgggtccgtctacccacccaacgaaggcttctgcccatgccgagagtctggcattcagaatgtcagcacctgcaggtttggtgcgcctctgtttctctcccacccccacttttacaacgccgaccctgtgttgtcagaagctgttcttggtctgaaccctaacccaaaggagcattccttgttcctagacatccatccggtcactgggatccccatgaactgttctgtgaagatgcagctgagcctctacatcaaatctgtcaagggcatcgggcaaacagggaagatcgagccagtagttctgccgttgctgtggttcgaacagagcggagcaatgggtggcaagcccctgagcacgttctacacgcagctggtgctgatgccccaggttcttcactacgcgcagtatgtgctgctggggcttggaggcctcctgttgctggtgcccatcatctgccaactgcgcagccaggagaaatgctttttgttttggagtggtagtaaaaagggctcccaggataaggaggccattcaggcctactctgagtccctgatgtcaccagctgccaagggcacggtgctgcaagaagccaagctatagggtcctgaagacactataagccccccaaacctgatagcttggtcagaccagccacccagtccctacaccccgcttcttgaggactctctcagcggacagcccaccagtgccatggcctgagcccccagatgtcacacctgtccgcacgcacggcacatggatgcccacgcatgtgcaaaaacaactcagggaccagggacagacctgctgccaagtgagcctgatgggccacaggtgtgctcttctaaatggcctgtgagccaggctgtgggaactctagctgctgtcagcccctcctgtaggagctggccctgcccaggctcctgacttccctcaggaagtctttctgtctttctccatcagtctgaaagccttagttcccacagaggacggatctgtcactcctaggggctgggcatatgtcggcctcttgtgccaaggccaggcaagcagctccaggtcctgaccagtttgcacacacactctggagctgtatctggcgctttttctatcgtctctgctatgtcactgaattaaccactgtacgtggcagaggtggcaggcccctcagggtccttatttttcaggcatggggtcaaagctagaggtatgggccgtctacacccccccgccccccggcatctagtgtacctcaccagagggtattcggaggcccagcatcctgcaaccgaccccttttttctactggaagagaaattttatcatcttttgaaaggaagtcatgactgaagcaataaaccttttcactgattcaacaaaaaaaaaaaaaaa

SEQ ID NO: 22 - DNA, 2759 bp, Homo sapiens
gctcaggccccgcccctgccgccggaatcctgaagcccaaggctgcccgggggcggtccggcggcgccggcgatggggcataaaaccactggccacctgccgggctgctcctgcgtgcgctgccgtcccggatccaccgtgcctctgcggcctgcgtgcccggagtccccgcctgtgtcgtctctgtcgccgtccccgtctcctgccaggcgcggagccctgcgagccgcgggtgggccccaggcgcgcagacatgggctgctccgccaaagcgcgctgggctgccggggcgctgggcgtcgcggggctactgtgcgctgtgctgggcgctgtcatgatcgtgatggtgccgtcgctcatcaagcagcaggtccttaagaacgtgcgcatcgaccccagtagcctgtccttcaacatgtggaaggagatccctatccccttctatctctccgtctacttctttgacgtcatgaaccccagcgagatcctgaagggcgagaagccgcaggtgcgggagcgcgggccctacgtgtacagggagttcaggcacaaaagcaacatcaccttcaacaacaacgacaccgtgtccttcctcgagtaccgcaccttccagttccagccctccaagtcccacggctcggagagcgactacatcgtcatgcccaacatcctggtcttgggtgcggcggtgatgatggagaataagcccatgaccctgaagctcatcatgaccttggcattcaccaccctcggcgaacgtgccttcatgaaccgcactgtgggtgagatcatgtggggctacaaggacccccttgtgaatctcatcaacaagtactttccaggcatgttccccttcaaggacaagttcggattatttgctgagctcaacaactccgactctgggctcttcacggtgttcacgggggtccagaacatcagcaggatccacctcgtggacaagtggaacgggctgagcaaggttgacttctggcattccgatcagtgcaacatgatcaatggaacttctgggcaaatgtggccgcccttcatgactcctgagtcctcgctggagttctacagcccggaggcctgccgatccatgaagctaatgtacaaggagtcaggggtgtttgaaggcatccccacctatcgcttcgtggctcccaaaaccctgtttgccaacgggtccatctacccacccaacgaaggcttctgcccgtgcctggagtctggaattcagaacgtcagcacctgcaggttcagtgcccccttgtttctctcccatcctcacttcctcaacgctgacccggttctggcagaagcggtgactggcctgcaccctaaccaggaggcacactccttgttcctggacatccacccggtcacgggaatccccatgaactgctctgtgaaactgcagctgagcctctacatgaaatctgtcgcaggcattggacaaactgggaagattgagcctgtggtcctgccgctgctctggtttgcagagagcggggccatggagggggagactcttcacacattctacactcagctggtgttgatgcccaaggtgatgcactatgcccagtacgtcctcctggcgctgggctgcgtcctgctgctggtccctgtcatctgccaaatccggagccaagagaaatgctatttattttggagtagtagtaaaaagggctcaaaggataaggaggccattcaggcctattctgaatccctgatgacatcagctcccaagggctctgtgctgcaggaagcaaaactgtagggtcctgaggacaccgtgagccagccaggcctggccgctgggcctgaccggccccccagcccctacaccccgcttctcccggactctcccagcggacagccccccagccccacagcctgagcctcccagctgccatgtgcctgttgcacacctgcacacacgccctggcacacatacacacatgcgtgcaggcttgtgcagacactcagggatggagctgctgctgaagggacttgtagggagaggctcgtcaacaagcactgttctggaaccttctctccacgtggcccacaggcctgaccacaggggctgtgggtcctgcgtccccttcctcgggtgagcctggcctgtcccgttcagccgttgggcccaggcttcctcccctccaaggtgaaacactgcagtcccggtgtggtggctccccatgcaggacgggccaggctgggagtgccgccttcctgtgccaaattcagtggggactcagtgcccaggccctggccacgagctttggccttggtctacctgccaggccaggcaaagcgcctttacacaggcctcggaaaacaatggagtgagcacaagatgccctgtgcagctgcccgagggtctccgcccaccccggccggactttgatccccccgaagtcttcacaggcactgcatcgggttgtctggcgcccttttcctccagcctaaactgacatcatcctatggactgagccggccactctctggccgaagtggccgcaggctgtgcccccgagctgcccccaccccctcacagggtccctcagattataggtgcccaggctgaggtgaagaggcctgggggccctgccttccgggcgctcctggaccctggggcaaacctgtgacccttttctactggaatagaaatgagttttatcatctttgaaaaataattcactcttgaagtaataaacgtttaaaaaaatgggaaaaaaaaaaaaaaaaaa

SEQ ID NO: 23 - DNA, 2761 bp, Mus musculus
gaactggccagagagacccaagggatagtcagggacgggcagacatgcagctagggttctggggcctggacaggggcagccaggccctgtgacgggaagaccccgagctccggcccggggaggggccatggtgttgcctgcccaacatgtcagccgaagtgcggctgaggcagctccagcagctggtgctggacccaggcttcctgggactggagcccctgctcgaccttctcctgggcgtccaccaggagctgggtgcctctcacctagcccaggacaagtatgtggccgacttcttgcagtgggtggagcccattgcagcaaggcttaaggaggtccgactgcagagggatgattttgagattttgaaggtgatcgggcgtggggcgttcagcgaggtagcggtggtgaagatgaaacagacgggccaagtgtatgccatgaagattatgaataagtgggacatgctgaagagaggcgaggtgtcgtgcttccgggaagaaagggatgtattagtgaaaggggaccggcgctggatcacacagctgcactttgccttccaggatgagaactacctgtacctggtcatggaatactacgtgggcggggacctgctaacgctgctgagcaagtttggggagcggatccccgccgagatggctcgcttctacctggccgagattgtcatggccatagactccgtgcaccggctgggctacgtgcacagggacatcaaaccagataacattctgctggaccgatgtgggcacattcgcctggcagacttcggctcctgcctcaaactgcagcctgatggaatggtgaggtcgctggtggctgtgggcaccccggactacctgtctcctgagattctgcaggccgttggtggagggcctggggcaggcagctacgggccagagtgtgactggtgggcactgggcgtgttcgcctatgagatgttctatgggcagacccccttctacgcggactccacagccgagacatatgccaagattgtgcactacagggaacacttgtcgctgccgctggcagacacagttgtccccgaggaagctcaggacctcattcgtgggctgctgtgtcctgctgagataaggctaggtcgaggtggggcaggtgatttccagaaacatcctttcttctttggccttgattgggagggtctccgagacagtgtacccccctttacaccagacttcgagggtgccacggacacatgcaatttcgatgtggtggaggaccggctcactgccatggtgagcgggggcggggagacgctgtcagacatgcaggaagacatgccccttggggtgcgcctgcccttcgtgggctactcctactgctgcatggccttcagagacaatcaggtcccggaccccacccctatggaactagaggccctgcagttgcctgtgtcagacttgcaagggcttgacttgcagcccccagtgtccccaccggatcaagtggctgaagaggctgacctagtggctgtccctgcccctgtggctgaggcagagaccacggtaacgctgcagcagctccaggaagccctggaagaagaggttctcacccggcagagcctgagccgcgagctggaggccatccggaccgccaaccagaacttctccagccaactacaggaggccgaggtccgaaaccgagacctggaggcgcatgttcggcagctacaggaacggatggagatgctgcaggccccaggagccgcagccatcacgggggtccccagtccccgggccacggatccaccttcccatctagatggccccccggccgtggctgtgggccagtgcccgctggtggggccaggccccatgcaccgccgtcacctgctgctccctgccaggatccctaggcctggcctatccgaggcgcgttgcctgctcctgttcgccgctgctctggctgctgccgccacactgggctgcactgggttggtggcctataccggcggtctcaccccagtctggtgtttcccgggagccaccttcgccccctgaaccctaagactccaagccatctttcatttaggcctcctaggaaggtcgagcgaccagggagcgacccaaagcgtctctgtgcccatcgcgccccccccccccccccaccgctccgctccacacttctgtgagcctgggtccccacccagctccgctcctgtgatccaggcctgccacctggcggccggggagggaggaacagggctcgtgcccagcacccctggttcctgcagagctggtagccaccgctgctgcagcagctgggcattcgccgaccttgctttactcagccccgacgtggatgggcaaactgctcagctcatccgatttcactttttcactctcccagccatcagttacaagccataagcatgagccccctatttccagggacatcccattcccatagtgatggatcagcaagacctctgccagcacacacggagtctttggcttcggacagcctcactcctgggggttgctgcaactccttccccgtgtacacgtctgcactctaacaacggagccacagctgcactcccccctcccccaaagcagtgtgggtatttattgatcttgttatctgactcactgacagactccgggacccacgttttagatgcattgagactcgacattcctcggtatttattgtctgtccccacctacgacctccactcccgacccttgcgaataaaatacttctggtctgccctaaa

SEQ ID NO: 24 - DNA, 3243 bp, Homo sapiens
gccacaagcctccaccccagctggtcccccacccaggctgcccagtttaacattcctagtcataggaccttgacttctgagaggcctgattgtcatctgtaaataaggggtaggactaaagcactcctcctggaggactgagagatgggctggaccggagcacttgagtctgggatatgtgaccatgctacctttgtctccctgtcctgttccttcccccagccccaaatccagggttttccaaagtgtggttcaagaaccacctgcatctgaatctagaggtactggatacaaccccacgtctgggccgttacccaggacattctacatgagaacgtgggggtggggccctggctgcacctgaactgtcacctggagtcagggtggaaggtggaagaactgggtcttatttccttctccccttgttctttagggtctgtccttctgcagactccgttaccccaccctaaccatcctgcacacccttggagccctctgggccaatgccctgtcccgcaaagggcttctcaggcatctcacctctatgggagggcatttttggcccccagaaccttacacggtgtttatgtggggaagcccctgggaagcagacagtcctagggtgaagctgagaggcagagagaaggggagacagacagagggtggggctttcccccttgtctccagtgccctttctggtgaccctcggttcttttcccccaccacccccccagcggagcccatcgtggtgaggcttaaggaggtccgactgcagagggacgacttcgagattctgaaggtgatcggacgcggggcgttcagcgaggtagcggtagtgaagatgaagcagacgggccaggtgtatgccatgaagatcatgaacaagtgggacatgctgaagaggggcgaggtgtcgtgcttccgtgaggagagggacgtgttggtgaatggggaccggcggtggatcacgcagctgcacttcgccttccaggatgagaactacctgtacctggtcatggagtattacgtgggcggggacctgctgacactgctgagcaagtttggggagcggattccggccgagatggcgcgcttctacctggcggagattgtcatggccatagactcggtgcaccggcttggctacgtgcacagggacatcaaacccgacaacatcctgctggaccgctgtggccacatccgcctggccgacttcggctcttgcctcaagctgcgggcagatggaacggtgcggtcgctggtggctgtgggcaccccagactacctgtcccccgagatcctgcaggctgtgggcggtgggcctgggacaggcagctacgggcccgagtgtgactggtgggcgctgggtgtattcgcctatgaaatgttctatgggcagacgcccttctacgcggattccacggcggagacctatggcaagatcgtccactacaaggagcacctctctctgccgctggtggacgaaggggtccctgaggaggctcgagacttcattcagcggttgctgtgtcccccggagacacggctgggccggggtggagcaggcgacttccggacacatcccttcttctttggcctcgactgggatggtctccgggacagcgtgcccccctttacaccggatttcgaaggtgccaccgacacatgcaacttcgacttggtggaggacgggctcactgccatggtgagcgggggcggggagacactgtcggacattcgggaaggtgcgccgctaggggtccacctgccttttgtgggctactcctactcctgcatggccctcagggacagtgaggtcccaggccccacacccatggaactggaggccgagcagctgcttgagccacacgtgcaagcgcccagcctggagccctcggtgtccccacaggatgaaacagctgaagtggcagttccagcggctgtccctgcggcagaggctgaggccgaggtgacgctgcgggagctccaggaagccctggaggaggaggtgctcacccggcagagcctgagccgggagatggaggccatccgcacggacaaccagaacttcgccagtcaactacgcgaggcagaggctcggaaccgggacctagaggcacacgtccggcagttgcaggagcggatggagttgctgcaggcagagggagccacagctgtcacgggggtccccagtccccgggccacggatccaccttcccatctagatggccccccggccgtggctgtgggccagtgcccgctggtggggccaggccccatgcaccgccgccacctgctgctccctgccagggtccctaggcctggcctatcggaggcgctttccctgctcctgttcgccgttgttctgtctcgtgccgccgccctgggctgcattgggttggtggcccacgccggccaactcaccgcagtctggcgccgcccaggagccgcccgcgctccctgaaccctagaactgtcttcgactccggggccccgttggaagactgagtgcccggggcacggcacagaagccgcgcccaccgcctgccagttcacaaccgctccgagcgtgggtctccgcccagctccagtcctgtgatccgggcccgccccctagcggccggggagggaggggccgggtccgcggccggcgaacggggctcgaagggtccttgtagccgggaatgctgctgctgctgctgctgctgctgctgctgctgctgctgctgctgctgctgctgctgctggggggatcacagaccatttctttctttcggccaggctgaggccctgacgtggatgggcaaactgcaggcctgggaaggcagcaagccgggccgtccgtgttccatcctccacgcacccccacctatcgttggttcgcaaagtgcaaagctttcttgtgcatgacgccctgctctggggagcgtctggcgcgatctctgcctgcttactcgggaaatttgcttttgccaaacccgctttttcggggatcccgcgcccccctcctcacttgcgctgctctcggagccccagccggctccgcccgcttcggcggtttggatatttattgacctcgtcctccgactcgctgacaggctacaggacccccaacaaccccaatccacgttttggatgcactgagaccccgacattcctcggtatttattgtctgtccccacctaggacccccacccccgaccctcgcgaataaaaggccctccatctgcccaaagctctgga